European Patent Specification EP 3 766 970 B1, published September 11, 2024. Title: Expression Vector Production & High-Throughput Cell Screening. Applicant: Kymab Limited. Application EP14772197.1 (PCT/GB2014/052836). The sequence listing filed with the application follows.

SEQUENCE LISTING (58 sequences)

SEQ ID NO: 1 - DNA, 28 bp, Homo sapiens
  Human heavy chain variable region-specific sequence.
tctagagaaaaccctgtgagcacagctc

SEQ ID NO: 2 - DNA, 24 bp, Homo sapiens
  Human heavy chain variable region-specific sequence.
gagaatcccctgagagctccgttc

SEQ ID NO: 3 - DNA, 24 bp, Homo sapiens
  Human heavy chain variable region-specific sequence.
tcagaagcccccagagcacaacgc

SEQ ID NO: 4 - DNA, 26 bp, Homo sapiens
  Human heavy chain variable region-specific sequence.
tgggagaatcccctagatcacagctc

SEQ ID NO: 5 - DNA, 24 bp, Homo sapiens
  Human heavy chain variable region-specific sequence.
acagaagcccccagagcgcagcac

SEQ ID NO: 6 - DNA, 24 bp, Homo sapiens
  Human heavy chain variable region-specific sequence.
cccaccatggacacactttgctcc

SEQ ID NO: 7 - DNA, 25 bp, Homo sapiens
  Human heavy chain variable region-specific sequence.
tggactccaaggcctttccacttgg

SEQ ID NO: 8 - DNA, 29 bp, Homo sapiens
  Human heavy chain variable region-specific sequence.
tggacctcctgcacaagaacatgaaacac

SEQ ID NO: 9 - DNA, 27 bp, Homo sapiens
  Human heavy chain variable region-specific sequence.
gcagtcaccagagctccagacaatgtc

SEQ ID NO: 10 - DNA, 29 bp, Homo sapiens
  Human heavy chain variable region-specific sequence.
aagaagaagcccctagaccacagctccac

SEQ ID NO: 11 - DNA, 26 bp, Homo sapiens
  Human heavy chain variable region-specific sequence.
tgagattcccaggtgtttccattcag

SEQ ID NO: 12 - DNA, 28 bp, Homo sapiens
  Human heavy chain variable region-specific sequence.
agagccccagccccagaattcccaggag

SEQ ID NO: 13 - DNA, 25 bp, Homo sapiens
  Human heavy chain variable region-specific sequence.
ttcagtgatcaggactgaacacaca

SEQ ID NO: 14 - DNA, 29 bp, Homo sapiens
  Human heavy chain variable region-specific sequence.
ccccagccttgggattcccaagtgttttc

SEQ ID NO: 15 - DNA, 26 bp, Homo sapiens
  Human heavy chain variable region-specific sequence.
tgagattcccacgtgtttccattcag

SEQ ID NO: 16 - DNA, 26 bp, Homo sapiens
  Human heavy chain variable region-specific sequence.
acttggtgatcagcacggagcaccga

SEQ ID NO: 17 - DNA, 27 bp, Homo sapiens
  Human heavy chain variable region-specific sequence.
ctgggattttcaggtgttttcatttgg

SEQ ID NO: 18 - DNA, 26 bp, Homo sapiens
  Human kappa chain variable region-specific sequence.
ggagtcagacccagtcaggacacagc

SEQ ID NO: 19 - DNA, 26 bp, Homo sapiens
  Human kappa chain variable region-specific sequence.
ggagtcagacccactcaggacacagc

SEQ ID NO: 20 - DNA, 26 bp, Homo sapiens
  Human kappa chain variable region-specific sequence.
ggaatcagtcccactcaggacacagc

SEQ ID NO: 21 - DNA, 26 bp, Homo sapiens
  Human kappa chain variable region-specific sequence.
ggagtcagtctcagtcaggacacagc

SEQ ID NO: 22 - DNA, 28 bp, Homo sapiens
  Human kappa chain variable region-specific sequence.
atcaggactcctcagttcaccttctcac

SEQ ID NO: 23 - DNA, 28 bp, Homo sapiens
  Human kappa chain variable region-specific sequence.
attaggactcctcaggtcaccttctcac

SEQ ID NO: 24 - DNA, 26 bp, Homo sapiens
  Human kappa chain variable region-specific sequence.
gaggaactgctcagttaggacccaga

SEQ ID NO: 25 - DNA, 25 bp, Homo sapiens
  Human kappa chain variable region-specific sequence.
gctacaacaggcaggcaggggcagc

SEQ ID NO: 26 - DNA, 27 bp, Homo sapiens
  Human kappa chain variable region-specific sequence.
gactaccacctgcaggtcagggccaag

SEQ ID NO: 27 - DNA, 21 bp, Homo sapiens
  Human kappa chain variable region-specific sequence.
atggcctggtctcctctcctc

SEQ ID NO: 28 - DNA, 21 bp, Homo sapiens
  Human kappa chain variable region-specific sequence.
atggccggcttccctctcctc

SEQ ID NO: 29 - DNA, 21 bp, Homo sapiens
  Human kappa chain variable region-specific sequence.
atgccctgggctctgctcctc

SEQ ID NO: 30 - DNA, 21 bp, Homo sapiens
  Human kappa chain variable region-specific sequence.
atgccctgggtcatgctcctc

SEQ ID NO: 31 - DNA, 21 bp, Homo sapiens
  Human kappa chain variable region-specific sequence.
atggcctgggctctgctgctc

SEQ ID NO: 32 - DNA, 21 bp, Homo sapiens
  Human kappa chain variable region-specific sequence.
atggcatggatccctctcttc

SEQ ID NO: 33 - DNA, 21 bp, Homo sapiens
  Human kappa chain variable region-specific sequence.
atggcctggacccctctcctg

SEQ ID NO: 34 - DNA, 21 bp, Homo sapiens
  Human kappa chain variable region-specific sequence.
atggcctggacccctctcctc

SEQ ID NO: 35 - DNA, 21 bp, Homo sapiens
  Human kappa chain variable region-specific sequence.
atggcctggacccctctctgg

SEQ ID NO: 36 - DNA, 21 bp, Homo sapiens
  Human kappa chain variable region-specific sequence.
atggcctggaccgttctcctc

SEQ ID NO: 37 - DNA, 21 bp, Homo sapiens
  Human kappa chain variable region-specific sequence.
atggcatgggccacactcctg

SEQ ID NO: 38 - DNA, 21 bp, Homo sapiens
  Human kappa chain variable region-specific sequence.
atggcctggatccctctactt

SEQ ID NO: 39 - DNA, 21 bp, Homo sapiens
  Human kappa chain variable region-specific sequence.
atggcctggatccctctcctg

SEQ ID NO: 40 - DNA, 21 bp, Homo sapiens
  Human kappa chain variable region-specific sequence.
atggcctggaccgctctcctt

SEQ ID NO: 41 - DNA, 21 bp, Homo sapiens
  Human kappa chain variable region-specific sequence.
atggcctgggtctccttctac

SEQ ID NO: 42 - DNA, 21 bp, Homo sapiens
  Human kappa chain variable region-specific sequence.
atggcctggaccccactcctc

SEQ ID NO: 43 - DNA, 21 bp, Homo sapiens
  Human kappa chain variable region-specific sequence.
atggcttggaccccactcctc

SEQ ID NO: 44 - DNA, 21 bp, Homo sapiens
  Human kappa chain variable region-specific sequence.
atggcctggactcctctcctc

SEQ ID NO: 45 - DNA, 21 bp, Homo sapiens
  Human kappa chain variable region-specific sequence.
atggcctggactcctctcttt

SEQ ID NO: 46 - DNA, 21 bp, Homo sapiens
  Human kappa chain variable region-specific sequence.
atggcctggatgatgcttctc

SEQ ID NO: 47 - DNA, 21 bp, Homo sapiens
  Human kappa chain variable region-specific sequence.
atggcctgggctcctctgctc

SEQ ID NO: 48 - DNA, 30 bp, Homo sapiens
  Human heavy chain constant region-specific sequence.
gctcttgcggtagcccttgaccaggcatcc

SEQ ID NO: 49 - DNA, 25 bp, Homo sapiens
  Human heavy chain constant region-specific sequence.
cagatccaggggccagtggatagac

SEQ ID NO: 50 - DNA, 35 bp, Homo sapiens
  Human kappa chain constant region-specific sequence.
gtttctgatcgaactaacactcattcctgttgaag

SEQ ID NO: 51 - DNA, 29 bp, Homo sapiens
  Human kappa chain constant region-specific sequence.
gacaatgggtgaagttgatgtcttgtgag

SEQ ID NO: 52 - DNA, 36 bp, Homo sapiens
  Human kappa chain constant region-specific sequence.
cgacaaccactacctctatgaacattctgtaggggc

SEQ ID NO: 53 - DNA, 25 bp, Homo sapiens
  Human kappa chain constant region-specific sequence.
cttctccacggtgctcccttcatgc

SEQ ID NO: 54 - DNA, 35 bp, Homo sapiens
  CMV promoter sequence
cttactggcttatcgaaattaatacgactcagatc

SEQ ID NO: 55 - DNA, 313 bp, Homo sapiens
  piggyBac (PB) transposon inverted 5' terminal repeat element
gatatctataacaagaaaatatatatataataagttatcacgtaagtagaacatgaaataacaatataattatcgtatgagttaaatcttaaaagtcacgtaaaagataatcatgcgtcattttgactcacgcggtcgttatagttcaaaatcagtgacacttaccgcattgacaagcacgcctcacgggagctccaagcggcgactgagatgtcctaaatgcacagcgacggattcgcgctatttagaaagagagagcaatatttcaagaatgcatgcgtcaattttacgcagactatctttctagggttaa

SEQ ID NO: 56 - DNA, 235 bp, Homo sapiens
  piggyBac (PB) transposon inverted 3' terminal repeat element
tttgttactttatagaagaaattttgagtttttgtttttttttaataaataaataaacataaataaattgtttgttgaatttattattagtatgtaagtgtaaatataataaaacttaatatctattcaaattaataaataaacctcgatatacagaccgataaaacacatgcgtcaattttacgcatgattatctttaacgtacgtcacaatatgattatctttctagggttaa

SEQ ID NO: 57 - protein, 594 aa, Homo sapiens
  Wildtype piggyBac transposase
MGCSLDDEHILSALLQSDDELVGEDSDSEISDHVSEDDVQSDTEEAFIDEVHEVQPTSSGSEILDEQNVIEQPGSSLASNRILTLPQRTIRGKNKHCWSTSKSTRRSRVSALNIVRSQRGPTRMCRNIYDPLLCFKLFFTDEIISEIVKWTNAEISLKRRESMTGATFRDTNEDEIYAFFGILVMTAVRKDNHMSTDDLFDRSLSMVYVSVMSRDRFDFLIRCLRMDDKSIRPTLRENDVFTPVRKIWDLFIHQCIQNYTPGAHLTIDEQLLGFRGRCPFRMYIPNKPSKYGIKILMMCDSGTKYMINGMPYLGRGTQTNGVPLGEYYVKELSKPVHGSCRNITCDNWFTSIPLAKNLLQEPYKLTIVGTVRSNKREIPEVLKNSRSRPVGTSMFCFDGPLTLVSYKPKPAKMVYLLSSCDEDASINESTGKPQMVMYYNQTKGGVDTLDQMCSVMTCSRKTNRWPMALLYGMINIACINSFIIYSHNVSSKGEKVQSRKKFMRNLYMSLTSSFMRKRLEAPTLKRYLRDNISNILPNEVPGTSDDSTEEPVMKKRTYCTYCPSKIRRKANASCKKCKKVICREHNIDMCQSCF

SEQ ID NO: 58 - protein, 594 aa, Homo sapiens
  Hyperactive piggyBac transposase
MGSSLDDEHILSALLQSDDELVGEDSDSEVSDHVSEDDVQSDTEEAFIDEVHEVQPTSSGSEILDEQNVIEQPGSSLASNRILTLPQRTIRGKNKHCWSTSKPTRRSRVSALNIVRSQRGPTRMCRNIYDPLLCFKLFFTDEIISEIVKWTNAEISLKRRESMTSATFRDTNEDEIYAFFGILVMTAVRKDNHMSTDDLFDRSLSMVYVSVMSRDRFDFLIRCLRMDDKSIRPTLRENDVFTPVRKIWDLFIHQCIQNYTPGAHLTIDEQLLGFRGRCPFRVYIPNKPSKYGIKILMMCDSGTKYMINGMPYLGRGTQTNGVPLGEYYVKELSKPVHGSCRNITCDNWFTSIPLAKNLLQEPYKLTIVGTVRSNKREIPEVLKNSRSRPVGTSMFCFDGPLTLVSYKPKPAKMVYLLSSCDEDASINESTGKPQMVMYYNQTKGGVDTLDQMCSVMTCSRKTNRWPMALLYGMINIACINSFIIYSHNVSSKGEKVQSRKKFMRNLYMGLTSSFMRKRLEAPTLKRYLRDNISNILPKEVPGTSDDSTEEPVMKKRTYCTYCPSKIRRKASASCKKCKKVICREHNIDMCQSCF